European Patent Application EP 4 663 757 A1, published December 17, 2025. Title: TAU splice-switching oligonucleotide and pharmaceutical composition for treating or preventing TAU-related disease. Applicant: OTSUKA PHARMACEUTICAL CO., LTD. The sequence listing filed with the application follows.

SEQUENCE LISTING (40 sequences)

SEQ ID NO: 1 - DNA, 135 bp, Homo sapiens
  source 1..135: mol_type = genomic DNA
aggggagtgaattcactgagctgagagctgaggaaccattgatctgatggctgagacaccactgggaagactggagaggcttttctgggcatgcagtgccaggcacaggaggagctgagggaagatgactaagag

SEQ ID NO: 2 - DNA, 2559 bp, Homo sapiens
  source 1..2559: mol_type = genomic DNA
gtactggcaaagaattcagaaattctgatggaagctttacatgttaccatcacatccatccatctatccacccatccatccacccatatcttcctccctccacccaatcatgcatacatccagtcatctatacaccacccacccacccatccatccatccatccatcccttcatccatcccatcatccatccaattatacatacatccaatcatatatctgtacataatccattcttccctcggttcatccatccatccattcatccatccatccacccatcccttccttcatccttcctatcatccatccaatcatatatctgtacataatccattcttccctcggttcatccatccatccattcatccatccatccacccatcccttccttcatccttcctatcatccatccaatcatacatatatccaatcatacatctgcacatcaccagctcatccatctatccatttatccatccatccttccttccatccatcattcatccatcatacatacatctaaccatacatctctacatcattcattcttccatcgattcatccaattatccatcattccttcctccatccatcccattatccatttgatcatacatatatcatctatacatcatccattcatccatccatccatccatccacccatatcttcatccaatcaatcatacatacatcgaatcatctacacatcacccatccatccatccatccattcatctatccacccatccatccatccatccatccattcatctatccacccatccatccatccatccatccatccatccatgtaaccatccagtcatatatccaattacacatccatccagttatacattcatacatgcatctaatcattcaattatacatacacacatccatataattctacatccaattatacctccatccaattacacattcatacacccacctaataaattattaattcatatatccatccatataattatacatcaattatacatccatctaatcattcagtaattcacccaccatccagtcatctatccaataatacattcatccaatcatccatccatccatccacccattcatccatccatccgtccgtccacccatcatggtatgagccatgatttaccacgatggtcccctgtggacagcccaggtggggcagaactgaagggaagcccagggctgcccccataaacatttgcctcctttacatggatgagaactagatccacatgtataaatcctcatgatttgaaggtgcttttaccaacattcactcatgggattctcccaggagctctaggaggaggcaggtagagttgaggtcatctcacgcattttacagatgaggaaacggaggccctgagaggcaggtccaaggccacctgaccagaaagaagtggaactgggacttgaacccagccatcttgccccttggtcccatgctctctagcctgtaactcctgcttcctggtggggcatctccaggaggaccctatcggctggccatgggcctgccctggagtcttttgctctgtgtggccatccttcctccctcaggagagtgtgtgctcccagagcacaggctgtatcttctgagcattttgtcccttcccagtacctagcactcagctctgtatacattgggctctcaagaattctcaaccttccagagtgtaaggccttgacctgctcagccctggatactgcatgatgcattgataagcccataaaataaccagggcagattgactcccagtggccaaagtgccacagggaagggacaattcagcccttctaggaggaggaggaggtagttttctcatttctattaaggcaacaaaagctgccttactaaggacattcttggtggagggcgtgactgtcaaccactgtgatcatttgggcctctcttgcccaggcttcccattctgaaaggacagttttattgtaggtacacatggctgccatttcaaatgtaactcacagcttgtccatcagtccttggaggtctttctatgaaaggagcttggtggcgtccaaacaccacccaatgtccacttagaagtaagcaccgtgtctgccctgagctgactccttttccaaggaaggggttggatcgctgagtgtttttccaggtgtctacttgttgttaattaatagcaatgacaaagcagaaggttcatgcgtagctcggctttctggtatttgctgcccgttgaccaatggaagataaacctttgcctcaggtggcaccactagctggttaagaggcactttgtcctttcacccaggagcaaacgcacatcacctgtgtcctcatctgatggccctggtgtggggcacagtcgtgttggcagggagggaggtggggttggtcccctttgtgggtttgttgcgaggccgtgttccagctgtttccacagggagcgattttcagctccacaggacactgctccccagttcctcctgagaacaaaagggggcgctggggagaggccaccgttctgagggctcactgtatgtgttccag

SEQ ID NO: 3 - DNA, 19 bp, Homo sapiens
  source 1..19: mol_type = genomic DNA
ggcaaagaattcagaaatt

SEQ ID NO: 4 - DNA, 18 bp, Homo sapiens
  source 1..18: mol_type = genomic DNA
ggcaaagaattcagaaat

SEQ ID NO: 5 - DNA, 18 bp, Homo sapiens
  source 1..18: mol_type = genomic DNA
gcaaagaattcagaaatt

SEQ ID NO: 6 - DNA, 18 bp, synthetic construct
  source 1..18: mol_type = other DNA
atttctgaattctttgcc

SEQ ID NO: 7 - DNA, 18 bp, synthetic construct
  source 1..18: mol_type = other DNA
aatttctgaattctttgc

SEQ ID NO: 8 - DNA, 18 bp, synthetic construct
  source 1..18: mol_type = other DNA
  modified_base 1..5: mod_base = OTHER; note = 2'-O-methoxyethyl nucleoside
  modified_base 14..18: mod_base = OTHER; note = 2'-O-methoxyethyl nucleoside
  modified_base 4: mod_base = m5c
  modified_base 12: mod_base = m5c
gggcgtatagacgtgtta

SEQ ID NO: 9 - DNA, 18 bp, synthetic construct
  source 1..18: mol_type = other DNA
  modified_base 1..5: mod_base = OTHER; note = 2'-O-methoxyethyl nucleoside
  modified_base 14..18: mod_base = OTHER; note = 2'-O-methoxyethyl nucleoside
  modified_base 1: mod_base = m5c
  modified_base 2: mod_base = m5c
  modified_base 8: mod_base = m5c
  modified_base 12: mod_base = m5c
  modified_base 13: mod_base = m5c
  modified_base 15: mod_base = m5c
  modified_base 16: mod_base = m5c
  modified_base 17: mod_base = m5c
ccgttttcttaccaccct

SEQ ID NO: 10 - DNA, 18 bp, synthetic construct
  source 1..18: mol_type = other DNA
  modified_base 1: mod_base = OTHER; note = Locked Nucleic Acid
  modified_base 3: mod_base = OTHER; note = Locked Nucleic Acid
  modified_base 5: mod_base = OTHER; note = Locked Nucleic Acid
  modified_base 7: mod_base = OTHER; note = Locked Nucleic Acid
  modified_base 9: mod_base = OTHER; note = Locked Nucleic Acid
  modified_base 11: mod_base = OTHER; note = Locked Nucleic Acid
  modified_base 13: mod_base = OTHER; note = Locked Nucleic Acid
  modified_base 15: mod_base = OTHER; note = Locked Nucleic Acid
  modified_base 17: mod_base = OTHER; note = Locked Nucleic Acid
  modified_base 3: mod_base = m5c
  modified_base 10: mod_base = m5c
  modified_base 15: mod_base = m5c
  modified_base 16: mod_base = m5c
ttctgaattctttgccag

SEQ ID NO: 11 - DNA, 18 bp, synthetic construct
  source 1..18: mol_type = other DNA
  modified_base 1: mod_base = OTHER; note = Locked Nucleic Acid
  modified_base 3: mod_base = OTHER; note = Locked Nucleic Acid
  modified_base 5: mod_base = OTHER; note = Locked Nucleic Acid
  modified_base 7: mod_base = OTHER; note = Locked Nucleic Acid
  modified_base 9: mod_base = OTHER; note = Locked Nucleic Acid
  modified_base 11: mod_base = OTHER; note = Locked Nucleic Acid
  modified_base 13: mod_base = OTHER; note = Locked Nucleic Acid
  modified_base 15: mod_base = OTHER; note = Locked Nucleic Acid
  modified_base 17: mod_base = OTHER; note = Locked Nucleic Acid
  modified_base 4: mod_base = m5c
  modified_base 11: mod_base = m5c
  modified_base 16: mod_base = m5c
  modified_base 17: mod_base = m5c
tttctgaattctttgcca

SEQ ID NO: 12 - DNA, 18 bp, synthetic construct
  source 1..18: mol_type = other DNA
  modified_base 1: mod_base = OTHER; note = Locked Nucleic Acid
  modified_base 3: mod_base = OTHER; note = Locked Nucleic Acid
  modified_base 5: mod_base = OTHER; note = Locked Nucleic Acid
  modified_base 7: mod_base = OTHER; note = Locked Nucleic Acid
  modified_base 9: mod_base = OTHER; note = Locked Nucleic Acid
  modified_base 11: mod_base = OTHER; note = Locked Nucleic Acid
  modified_base 13: mod_base = OTHER; note = Locked Nucleic Acid
  modified_base 15: mod_base = OTHER; note = Locked Nucleic Acid
  modified_base 17: mod_base = OTHER; note = Locked Nucleic Acid
  modified_base 5: mod_base = m5c
  modified_base 12: mod_base = m5c
  modified_base 17: mod_base = m5c
  modified_base 18: mod_base = m5c
atttctgaattctttgcc

SEQ ID NO: 13 - DNA, 18 bp, synthetic construct
  source 1..18: mol_type = other DNA
  modified_base 1: mod_base = OTHER; note = Locked Nucleic Acid
  modified_base 3: mod_base = OTHER; note = Locked Nucleic Acid
  modified_base 5: mod_base = OTHER; note = Locked Nucleic Acid
  modified_base 7: mod_base = OTHER; note = Locked Nucleic Acid
  modified_base 9: mod_base = OTHER; note = Locked Nucleic Acid
  modified_base 11: mod_base = OTHER; note = Locked Nucleic Acid
  modified_base 13: mod_base = OTHER; note = Locked Nucleic Acid
  modified_base 15: mod_base = OTHER; note = Locked Nucleic Acid
  modified_base 17: mod_base = OTHER; note = Locked Nucleic Acid
  modified_base 6: mod_base = m5c
  modified_base 13: mod_base = m5c
  modified_base 18: mod_base = m5c
aatttctgaattctttgc

SEQ ID NO: 14 - DNA, 18 bp, synthetic construct
  source 1..18: mol_type = other DNA
  modified_base 1: mod_base = OTHER; note = Locked Nucleic Acid
  modified_base 3: mod_base = OTHER; note = Locked Nucleic Acid
  modified_base 5: mod_base = OTHER; note = Locked Nucleic Acid
  modified_base 7: mod_base = OTHER; note = Locked Nucleic Acid
  modified_base 9: mod_base = OTHER; note = Locked Nucleic Acid
  modified_base 11: mod_base = OTHER; note = Locked Nucleic Acid
  modified_base 13: mod_base = OTHER; note = Locked Nucleic Acid
  modified_base 15: mod_base = OTHER; note = Locked Nucleic Acid
  modified_base 17: mod_base = OTHER; note = Locked Nucleic Acid
  modified_base 7: mod_base = m5c
  modified_base 14: mod_base = m5c
gaatttctgaattctttg

SEQ ID NO: 15 - DNA, 18 bp, synthetic construct
  source 1..18: mol_type = other DNA
  modified_base 1: mod_base = OTHER; note = Locked Nucleic Acid
  modified_base 3: mod_base = OTHER; note = Locked Nucleic Acid
  modified_base 5: mod_base = OTHER; note = Locked Nucleic Acid
  modified_base 7: mod_base = OTHER; note = Locked Nucleic Acid
  modified_base 9: mod_base = OTHER; note = Locked Nucleic Acid
  modified_base 11: mod_base = OTHER; note = Locked Nucleic Acid
  modified_base 13: mod_base = OTHER; note = Locked Nucleic Acid
  modified_base 15: mod_base = OTHER; note = Locked Nucleic Acid
  modified_base 17: mod_base = OTHER; note = Locked Nucleic Acid
  modified_base 8: mod_base = m5c
  modified_base 15: mod_base = m5c
agaatttctgaattcttt

SEQ ID NO: 16 - DNA, 18 bp, synthetic construct
  source 1..18: mol_type = other DNA
  modified_base 1: mod_base = OTHER; note = Amido-Bridged Nucleic Acid
  modified_base 3: mod_base = OTHER; note = Amido-Bridged Nucleic Acid
  modified_base 5: mod_base = OTHER; note = Amido-Bridged Nucleic Acid
  modified_base 7: mod_base = OTHER; note = Amido-Bridged Nucleic Acid
  modified_base 9: mod_base = OTHER; note = Amido-Bridged Nucleic Acid
  modified_base 11: mod_base = OTHER; note = Amido-Bridged Nucleic Acid
  modified_base 13: mod_base = OTHER; note = Amido-Bridged Nucleic Acid
  modified_base 15: mod_base = OTHER; note = Amido-Bridged Nucleic Acid
  modified_base 17: mod_base = OTHER; note = Amido-Bridged Nucleic Acid
  modified_base 5: mod_base = m5c
  modified_base 12: mod_base = m5c
  modified_base 17: mod_base = m5c
  modified_base 18: mod_base = m5c
atttctgaattctttgcc

SEQ ID NO: 17 - DNA, 18 bp, synthetic construct
  source 1..18: mol_type = other DNA
  modified_base 1: mod_base = OTHER; note = Amido-Bridged Nucleic Acid
  modified_base 3: mod_base = OTHER; note = Amido-Bridged Nucleic Acid
  modified_base 5: mod_base = OTHER; note = Amido-Bridged Nucleic Acid
  modified_base 7: mod_base = OTHER; note = Amido-Bridged Nucleic Acid
  modified_base 9: mod_base = OTHER; note = Amido-Bridged Nucleic Acid
  modified_base 11: mod_base = OTHER; note = Amido-Bridged Nucleic Acid
  modified_base 13: mod_base = OTHER; note = Amido-Bridged Nucleic Acid
  modified_base 15: mod_base = OTHER; note = Amido-Bridged Nucleic Acid
  modified_base 17: mod_base = OTHER; note = Amido-Bridged Nucleic Acid
  modified_base 6: mod_base = m5c
  modified_base 13: mod_base = m5c
  modified_base 18: mod_base = m5c
aatttctgaattctttgc

SEQ ID NO: 18 - DNA, 20 bp, synthetic construct
  source 1..20: mol_type = other DNA
catgcaccaagaccaagagg

SEQ ID NO: 19 - DNA, 19 bp, synthetic construct
  source 1..19: mol_type = other DNA
tcacgtgaccagcagcttc

SEQ ID NO: 20 - DNA, 17 bp, synthetic construct
  source 1..17: mol_type = other DNA
acagagcctcgcctttg

SEQ ID NO: 21 - DNA, 17 bp, synthetic construct
  source 1..17: mol_type = other DNA
ccttgcacatgccggag

SEQ ID NO: 22 - DNA, 259 bp, synthetic construct
  source 1..259: mol_type = other DNA
tcaggggggctacaccatgcaccaagaccaagagggtgacacggacgctggcctgaaagaggggagtgaattcactgagctgagagctgaggaaccattgatctgatggctgagacaccactgggaagactggagaggcttttctgggcatgcagtgccaggcacaggaggagctgagggaagatgactaagagctgaagaagcaggcattggagacacccccagcctggaagacgaagctgctggtcacgtgacccaa

SEQ ID NO: 23 - DNA, 125 bp, synthetic construct
  source 1..125: mol_type = other DNA
tcaggggggctacaccatgcaccaagaccaagagggtgacacggacgctggcctgaaagctgaagaagcaggcattggagacacccccagcctggaagacgaagctgctggtcacgtgacccaag

SEQ ID NO: 24 - DNA, 366 bp, synthetic construct
  source 1..366: mol_type = other DNA
gcatcgacatcgactaaccgccgagaccgcgtccgccccgcgagcacagagcctcgcctttgccgatccgccgcccgtccacacccgccgccagctcaccatggatgatgatatcgccgcgctcgtcgtcgacaacggctccggcatgtgcaaggccggcttcgcgggcgacgatgccccccgggccgtcttcccctccatcgtggggcgccccaggcaccagggcgtgatggtgggcatgggtcagaaggattcctatgtgggcgacgaggcccagagcaagagaggcatcctcaccctgaagtaccccatcgagcacggcatcgtcaccaactgggacgacatggagaaaatctggcaccacac

SEQ ID NO: 25 - DNA, 23 bp, synthetic construct
  source 1..23: mol_type = other DNA
caggctttacactttatgcttcc

SEQ ID NO: 26 - DNA, 20 bp, synthetic construct
  source 1..20: mol_type = other DNA
cgatttcggcctattggtta

SEQ ID NO: 27 - DNA, 125 bp, synthetic construct
  source 1..125: mol_type = other DNA
tctagtaaacaataactgtcttgcttttaccccccttcatttgctgacacatacaccagctgaagaagcaggcattggagacacccccagcctggaagacgaagctgctggtcacgtgacccaag

SEQ ID NO: 28 - DNA, 22 bp, synthetic construct
  source 1..22: mol_type = other DNA
agggaagatgactaagagctga

SEQ ID NO: 29 - DNA, 18 bp, synthetic construct
  source 1..18: mol_type = other DNA
tcacgtgaccagcagctt

SEQ ID NO: 30 - DNA, 21 bp, synthetic construct
  source 1..21: mol_type = other DNA
agacacccccagcctggaaga

SEQ ID NO: 31 - DNA, 17 bp, synthetic construct
  source 1..17: mol_type = other DNA
gctggcctgaaagctga

SEQ ID NO: 32 - DNA, 23 bp, synthetic construct
  source 1..23: mol_type = other DNA
cttcatttgctgacacatacacc

SEQ ID NO: 33 - DNA, 21 bp, synthetic construct
  source 1..21: mol_type = other DNA
tcatccatggtgagctggcgg

SEQ ID NO: 34 - DNA, 19 bp, synthetic construct
  source 1..19: mol_type = other DNA
ccatcagcaacgacctcaa

SEQ ID NO: 35 - DNA, 19 bp, synthetic construct
  source 1..19: mol_type = other DNA
gcttccaggaccttgttct

SEQ ID NO: 36 - DNA, 21 bp, synthetic construct
  source 1..21: mol_type = other DNA
cttcgccagcttcatcgagcg

SEQ ID NO: 37 - DNA, 178 bp, synthetic construct
  source 1..178: mol_type = other DNA
cgacctgagccaggtagccgccatcagcaacgacctcaagtccatccgcacgcaggagaaggcgcagctccaggacctcaatgaccgcttcgccagcttcatcgagcgcgtgcacgagctggagcagcagaacaaggtcctggaagccgagctgctggtgctgcgccagaagcactcc

SEQ ID NO: 38 - DNA, 37 bp, Homo sapiens
  source 1..37: mol_type = genomic DNA
gaggtactggcaaagaattcagaaattctgatggaag

SEQ ID NO: 39 - DNA, 18 bp, synthetic construct
  source 1..18: mol_type = other DNA
  modified_base 1..4: mod_base = OTHER; note = Locked Nucleic Acid
  modified_base 15..18: mod_base = OTHER; note = Locked Nucleic Acid
atttctgaattctttgcc

SEQ ID NO: 40 - DNA, 18 bp, synthetic construct
  source 1..18: mol_type = other DNA
  modified_base 1..4: mod_base = OTHER; note = Locked Nucleic Acid
  modified_base 15..18: mod_base = OTHER; note = Locked Nucleic Acid
aatttctgaattctttgc